European Patent Application EP 4 474 387 A1, published December 11, 2024. Title: オリゴヌクレオチドを製造する方法. Applicant: 日東電工株式会社. Application JP. The sequence listing filed with the application follows.

SEQUENCE LISTING (2 sequences)

SEQ ID NO: 1 - DNA, 24 bp, synthetic construct
  source 1..24: mol_type = other DNA
tcgacgtattgacgtattgacgta

SEQ ID NO: 2 - RNA, 24 nt, synthetic construct
  source 1..24: mol_type = other RNA
  modified_base 1: mod_base = um
  modified_base 2: mod_base = cm
  modified_base 3: mod_base = gm
  modified_base 4: mod_base = OTHER; note = 2'-O-methyladenosine
  modified_base 5: mod_base = cm
  modified_base 6: mod_base = gm
  modified_base 7: mod_base = um
  modified_base 8: mod_base = OTHER; note = 2'-O-methyladenosine
  modified_base 9..10: mod_base = um
  modified_base 11: mod_base = gm
  modified_base 12: mod_base = OTHER; note = 2'-O-methyladenosine
  modified_base 13: mod_base = cm
  modified_base 14: mod_base = gm
  modified_base 15: mod_base = um
  modified_base 16: mod_base = OTHER; note = 2'-O-methyladenosine
  modified_base 17..18: mod_base = um
  modified_base 19: mod_base = gm
  modified_base 20: mod_base = OTHER; note = 2'-O-methyladenosine
  modified_base 21: mod_base = cm
  modified_base 22: mod_base = gm
  modified_base 23: mod_base = um
  modified_base 24: mod_base = OTHER; note = 2'-O-methyladenosine
tcgacgtattgacgtattgacgta